European Patent Specification EP 3 740 499 B1, published May 14, 2025. Title: Novel anti-tumor therapeutic agents. Applicant: Università degli Studi del Piemonte Orientale "Amedeo Avogadro" NOVAICOS SRLS. The sequence listing filed with the application follows.

SEQUENCE LISTING (24 sequences)

SEQ ID NO: 1 - protein, 199 aa, homo sapiens
MKSGLWYFFLFCLRIKVLTGEINGSANYEMFIFHNGGVQILCKYPDIVQQFKMQLLKGGQILCDLTKTKGSGNTVSIKSLKFCHSQLSNNSVSFFLYNLDHSHANYYFCNLSIFDPPPFKVTLTGGYLHIYESQLCCQLKFWLPIGCAAFVVVCILGCILICWLTKKKYSSSVHDPNGEYMFMRAVNTAKKSRLTDVTL

SEQ ID NO: 2 - protein, 115 aa, homo sapiens
EINGSANYEMFIFHNGGVQILCKYPDIVQQFKMQLLKGGQILCDLTKTKGSGNTVSIKSLKFCHSQLSNNSVSFFLYNLDHSHANYYFCNLSIFDPPPFKVTLTGGYLHIYESQL

SEQ ID NO: 3 - protein, 348 aa, artificial
  human ICOS-Human Fc
GAHGEINGSANYEMFIFHNGGVQILCKYPDIVQQFKMQLLKGGQILCDLTKTKGSGNTVSIKSLKFCHSQLSNNSVSFFLYNLDHSHANYYFCNLSIFDPPPFKVTLTGGYLHIYESQLASDKTHTCPPCPAPELLGGPSVFLFPPKPKDTLMISRTPEVTCVVVDVSHEDPEVKFNWYVDGVEVHNAKTKPREEQYNSTYRVVSVLTVLHQDWLNGKEYKCKVSNKALPAPIEKTISKAKGQPREPQVYTLPPSREEMTKNQVSLTCLVKGFYPSDIAVEWESNGQPENNYKTTPPVLDSDGSFFLYSKLTVDKSRWQQGNVFSCSVMHEALHNHYTQKSLSLSPGK

SEQ ID NO: 4 - DNA, 345 bp, homo sapiens
gaaatcaatggttctgccaattatgagatgtttatatttcacaacggaggtgtacaaattttatgcaaatatcctgacattgtccagcaatttaaaatgcagttgctgaaaggggggcaaatactctgcgatctcactaagacaaaaggaagtggaaacacagtgtccattaagagtctgaaattctgccattctcagttatccaacaacagtgtctctttttttctatacaacttggaccattctcatgccaactattacttctgcaacctatcaatttttgatcctcctccttttaaagtaactcttacaggaggatatttgcatatttatgaatcacaactt

SEQ ID NO: 5 - DNA, 681 bp, homo sapiens
gacaaaactcacacatgcccaccgtgcccagcacctgaactcctggggggaccgtcagtcttcctcttccccccaaaacccaaggacaccctcatgatctcccggacccctgaggtcacatgcgtggtggtggacgtgagccacgaagaccctgaggtcaagttcaactggtacgtggacggcgtggaggtgcataatgccaagacaaagccgcgggaggagcagtacaacagcacgtaccgtgtggtcagcgtcctcaccgtcctgcaccaggactggctgaatggcaaggagtacaagtgcaaggtctccaacaaagccctcccagcccccatcgagaaaaccatctccaaagccaaagggcagccccgagaaccacaggtgtacaccctgcccccatcccgggaggagatgaccaagaaccaggtcagcctgacctgcctggtcaaaggcttctatcccagcgacatcgccgtggagtgggagagcaatgggcagccggagaacaactacaagaccacgcctcccgtgctggactccgacggctccttcttcctctatagcaagctcaccgtggacaagagcaggtggcagcaggggaacgtcttctcatgctccgtgatgcatgaggctctgcacaaccactacacgcagaagagcctctccctgtccccgggtaaa

SEQ ID NO: 6 - DNA, 6729 bp, artificial
  vector encoding huICOS-huFc
gacggatcgggagatctcccgatcccctatggtgcactctcagtacaatctgctctgatgccgcatagttaagccagtatctgctccctgcttgtgtgttggaggtcgctgagtagtgcgcgagcaaaatttaagctacaacaaggcaaggcttgaccgacaattgcatgaagaatctgcttagggttaggcgttttgcgctgcttcgcgatgtacgggccagatatacgcgttgacattgattattgactagttattaatagtaatcaattacggggtcattagttcatagcccatatatggagttccgcgttacataacttacggtaaatggcccgcctggctgaccgcccaacgacccccgcccattgacgtcaataatgacgtatgttcccatagtaacgccaatagggactttccattgacgtcaatgggtggagtatttacggtaaactgcccacttggcagtacatcaagtgtatcatatgccaagtacgccccctattgacgtcaatgacggtaaatggcccgcctggcattatgcccagtacatgaccttatgggactttcctacttggcagtacatctacgtattagtcatcgctattaccatggtgatgcggttttggcagtacatcaatgggcgtggatagcggtttgactcacggggatttccaagtctccaccccattgacgtcaatgggagtttgttttggcaccaaaatcaacgggactttccaaaatgtcgtaacaactccgccccattgacgcaaatgggcggtaggcgtgtacggtgggaggtctatataagcagagctctctggctaactagagaacccactgcttactggcttatcgaaattaatacgactcactatagggagacccaagctgtctagatgccaccatgggctggagcctgatcctcctgttcctcgtcgctgtggctacaggtaaggggctcacagtagcaggcttgaggtctggacatatatatgggtgacaatgacatccactttgcctttctctccacaggtggcgcgcatgccgaaatcaatggttctgccaattatgagatgtttatatttcacaacggaggtgtacaaattttatgcaaatatcctgacattgtccagcaatttaaaatgcagttgctgaaaggggggcaaatactctgcgatctcactaagacaaaaggaagtggaaacacagtgtccattaagagtctgaaattctgccattctcagttatccaacaacagtgtctctttttttctatacaacttggaccattctcatgccaactattacttctgcaacctatcaatttttgatcctcctccttttaaagtaactcttacaggaggatatttgcatatttatgaatcacaacttgctagcgacaaaactcacacatgcccaccgtgcccagcacctgaactcctggggggaccgtcagtcttcctcttccccccaaaacccaaggacaccctcatgatctcccggacccctgaggtcacatgcgtggtggtggacgtgagccacgaagaccctgaggtcaagttcaactggtacgtggacggcgtggaggtgcataatgccaagacaaagccgcgggaggagcagtacaacagcacgtaccgtgtggtcagcgtcctcaccgtcctgcaccaggactggctgaatggcaaggagtacaagtgcaaggtctccaacaaagccctcccagcccccatcgagaaaaccatctccaaagccaaagggcagccccgagaaccacaggtgtacaccctgcccccatcccgggaggagatgaccaagaaccaggtcagcctgacctgcctggtcaaaggcttctatcccagcgacatcgccgtggagtgggagagcaatgggcagccggagaacaactacaagaccacgcctcccgtgctggactccgacggctccttcttcctctatagcaagctcaccgtggacaagagcaggtggcagcaggggaacgtcttctcatgctccgtgatgcatgaggctctgcacaaccactacacgcagaagagcctctccctgtccccgggtaaaactagtggcaaaccaatcccaaacccactgctgggcctggatagtacttaaaagcttaaacccgctgatcagcctcgactgtgccttctagttgccagccatctgttgtttgcccctcccccgtgccttccttgaccctggaaggtgccactcccactgtcctttcctaataaaatgaggaaattgcatcgcattgtctgagtaggtgtcattctattctggggggtggggtggggcaggacagcaagggggaggattgggaagacaatagcaggcatgctggggatgcggtgggctctatggcttctgaggcggaaagaaccagctggggctctagggggtatccccacgcgccctgtagcggcgcattaagcgcggcgggtgtggtggttacgcgcagcgtgaccgctacacttgccagcgccctagcgcccgctcctttcgctttcttcccttcctttctcgccacgttcgccggctttccccgtcaagctctaaatcgggggctccctttagggttccgatttagtgctttacggcacctcgaccccaaaaaacttgattagggtgatggttcacgtagtgggccatcgccctgatagacggtttttcgccctttgacgttggagtccacgttctttaatagtggactcttgttccaaactggaacaacactcaaccctatctcggtctattcttttgatttataagggattttgccgatttcggcctattggttaaaaaatgagctgatttaacaaaaatttaacgcgaattaattctgtggaatgtgtgtcagttagggtgtggaaagtccccaggctccccagcaggcagaagtatgcaaagcatgcatctcaattagtcagcaaccaggtgtggaaagtccccaggctccccagcaggcagaagtatgcaaagcatgcatctcaattagtcagcaaccatagtcccgcccctaactccgcccatcccgcccctaactccgcccagttccgcccattctccgccccatggctgactaattttttttatttatgcagaggccgaggccgcctctgcctctgagctattccagaagtagtgaggaggcttttttggaggcctaggcttttgcaaaaagctcccgggagcttgtatatccattttcggatctgatcagcacgtgatgaaaaagcctgaactcaccgcgacgtctgtcgagaagtttctgatcgaaaagttcgacagcgtctccgacctgatgcagctctcggagggcgaagaatctcgtgctttcagcttcgatgtaggagggcgtggatatgtcctgcgggtaaatagctgcgccgatggtttctacaaagatcgttatgtttatcggcactttgcatcggccgcgctcccgattccggaagtgcttgacattggggaattcagcgagagcctgacctattgcatctcccgccgtgcacagggtgtcacgttgcaagacctgcctgaaaccgaactgcccgctgttctgcagccggtcgcggaggccatggatgcgatcgctgcggccgatcttagccagacgagcgggttcggcccattcggaccgcaaggaatcggtcaatacactacatggcgtgatttcatatgcgcgattgctgatccccatgtgtatcactggcaaactgtgatggacgacaccgtcagtgcgtccgtcgcgcaggctctcgatgagctgatgctttgggccgaggactgccccgaagtccggcacctcgtgcacgcggatttcggctccaacaatgtcctgacggacaatggccgcataacagcggtcattgactggagcgaggcgatgttcggggattcccaatacgaggtcgccaacatcttcttctggaggccgtggttggcttgtatggagcagcagacgcgctacttcgagcggaggcatccggagcttgcaggatcgccgcggctccgggcgtatatgctccgcattggtcttgaccaactctatcagagcttggttgacggcaatttcgatgatgcagcttgggcgcagggtcgatgcgacgcaatcgtccgatccggagccgggactgtcgggcgtacacaaatcgcccgcagaagcgcggccgtctggaccgatggctgtgtagaagtactcgccgatagtggaaaccgacgccccagcactcgtccgagggcaaaggaatagcacgtgctacgagatttcgattccaccgccgccttctatgaaaggttgggcttcggaatcgttttccgggacgccggctggatgatcctccagcgcggggatctcatgctggagttcttcgcccaccccaacttgtttattgcagcttataatggttacaaataaagcaatagcatcacaaatttcacaaataaagcatttttttcactgcattctagttgtggtttgtccaaactcatcaatgtatcttatcatgtctgtataccgtcgacctctagctagagcttggcgtaatcatggtcatagctgtttcctgtgtgaaattgttatccgctcacaattccacacaacatacgagccggaagcataaagtgtaaagcctggggtgcctaatgagtgagctaactcacattaattgcgttgcgctcactgcccgctttccagtcgggaaacctgtcgtgccagctgcattaatgaatcggccaacgcgcggggagaggcggtttgcgtattgggcgctcttccgcttcctcgctcactgactcgctgcgctcggtcgttcggctgcggcgagcggtatcagctcactcaaaggcggtaatacggttatccacagaatcaggggataacgcaggaaagaacatgtgagcaaaaggccagcaaaaggccaggaaccgtaaaaaggccgcgttgctggcgtttttccataggctccgcccccctgacgagcatcacaaaaatcgacgctcaagtcagaggtggcgaaacccgacaggactataaagataccaggcgtttccccctggaagctccctcgtgcgctctcctgttccgaccctgccgcttaccggatacctgtccgcctttctcccttcgggaagcgtggcgctttctcatagctcacgctgtaggtatctcagttcggtgtaggtcgttcgctccaagctgggctgtgtgcacgaaccccccgttcagcccgaccgctgcgccttatccggtaactatcgtcttgagtccaacccggtaagacacgacttatcgccactggcagcagccactggtaacaggattagcagagcgaggtatgtaggcggtgctacagagttcttgaagtggtggcctaactacggctacactagaagaacagtatttggtatctgcgctctgctgaagccagttaccttcggaaaaagagttggtagctcttgatccggcaaacaaaccaccgctggtagcggtttttttgtttgcaagcagcagattacgcgcagaaaaaaaggatctcaagaagatcctttgatcttttctacggggtctgacgctcagtggaacgaaaactcacgttaagggattttggtcatgagattatcaaaaaggatcttcacctagatccttttaaattaaaaatgaagttttaaatcaatctaaagtatatatgagtaaacttggtctgacagttaccaatgcttaatcagtgaggcacctatctcagcgatctgtctatttcgttcatccatagttgcctgactccccgtcgtgtagataactacgatacgggagggcttaccatctggccccagtgctgcaatgataccgcgagacccacgctcaccggctccagatttatcagcaataaaccagccagccggaagggccgagcgcagaagtggtcctgcaactttatccgcctccatccagtctattaattgttgccgggaagctagagtaagtagttcgccagttaatagtttgcgcaacgttgttgccattgctacaggcatcgtggtgtcacgctcgtcgtttggtatggcttcattcagctccggttcccaacgatcaaggcgagttacatgatcccccatgttgtgcaaaaaagcggttagctccttcggtcctccgatcgttgtcagaagtaagttggccgcagtgttatcactcatggttatggcagcactgcataattctcttactgtcatgccatccgtaagatgcttttctgtgactggtgagtactcaaccaagtcattctgagaatagtgtatgcggcgaccgagttgctcttgcccggcgtcaatacgggataataccgcgccacatagcagaactttaaaagtgctcatcattggaaaacgttcttcggggcgaaaactctcaaggatcttaccgctgttgagatccagttcgatgtaacccactcgtgcacccaactgatcttcagcatcttttactttcaccagcgtttctgggtgagcaaaaacaggaaggcaaaatgccgcaaaaaagggaataagggcgacacggaaatgttgaatactcatactcttcctttttcaatattattgaagcatttatcagggttattgtctcatgagcggatacatatttgaatgtatttagaaaaataaacaaataggggttccgcgcacatttccccgaaaagtgccacctgacgtc

SEQ ID NO: 7 - protein, 352 aa, artificial
  msICOS-msFc
GAHGEINGSADHRMFSFHNGGVQISCKYPETVQQLKMRLFREREVLCELTKTKGSGNAVSIKNPMLCLYHLSNNSVSFFLNNPDSSQGSYYFCSLSIFDPPPFQERNLSGGYLHIYESQLCCQLKLWLASGCKPCICTVPEVSSVFIFPPKPKDVLTITLTPKVTCVVVDISKDDPEVQFSWFVDDVEVHTAQTKPREEQINSTFRSVSELPIMHQDWLNGKEFKCRVNSAAFPAPIEKTISKTKGRPKAPQVYTIPPPKEQMAKDKVSLTCMITNFFPEDITVEWQWNGQPAENYKNTQPIMDTDGSYFVYSKLNVQKSNWEAGNTFTCSVLHEGLHNHHTEKSLSHSPGK

SEQ ID NO: 8 - DNA, 372 bp, mus musculus
gaaatcaatggctcggccgatcataggatgttttcatttcacaatggaggtgtacagatttcttgtaaataccctgagactgtccagcagttaaaaatgcgattgttcagagagagagaagtcctctgcgaactcaccaagaccaagggaagcggaaatgcggtgtccatcaagaatccaatgctctgtctatatcatctgtcaaacaacagcgtctcttttttcctaaacaacccagacagctcccagggaagctattacttctgcagcctgtccatttttgacccacctccttttcaagaaaggaaccttagtggaggatatttgcatatttatgaatcccagctctgctgccagctgaagctctggcta

SEQ ID NO: 9 - DNA, 666 bp, mus musculus
ggttgtaagccttgcatatgtacagtcccagaagtatcatctgtcttcatcttccccccaaagcccaaggatgtgctcaccattactctgactcctaaggtcacgtgtgttgtggtagacatcagcaaggatgatcccgaggtccagttcagctggtttgtagatgatgtggaggtgcacacagctcagacgaaaccccgggaggagcagatcaacagcactttccgttcagtcagtgaacttcccatcatgcaccaggactggctcaatggcaaggagttcaaatgcagggtcaacagtgcagctttccctgcccccatcgagaaaaccatctccaaaaccaaaggcagaccgaaggctccacaggtgtacaccattccacctcccaaggagcagatggccaaggataaagtcagtctgacctgcatgataacaaacttcttccctgaagacattactgtggagtggcagtggaatgggcagccagcggagaactacaagaacactcagcccatcatggacacagatggctcttacttcgtctacagcaagctcaatgtgcagaagagcaactgggaggcaggaaatactttcacctgctctgtgttacatgagggcctgcacaaccaccatactgagaagagcctctcccactctcctggtaaa

SEQ ID NO: 10 - DNA, 6719 bp, artificial
  vector encoding msICOS-msFc contruct
gacggatcgggagatctcccgatcccctatggtgcactctcagtacaatctgctctgatgccgcatagttaagccagtatctgctccctgcttgtgtgttggaggtcgctgagtagtgcgcgagcaaaatttaagctacaacaaggcaaggcttgaccgacaattgcatgaagaatctgcttagggttaggcgttttgcgctgcttcgcgatgtacgggccagatatacgcgttgacattgattattgactagttattaatagtaatcaattacggggtcattagttcatagcccatatatggagttccgcgttacataacttacggtaaatggcccgcctggctgaccgcccaacgacccccgcccattgacgtcaataatgacgtatgttcccatagtaacgccaatagggactttccattgacgtcaatgggtggagtatttacggtaaactgcccacttggcagtacatcaagtgtatcatatgccaagtacgccccctattgacgtcaatgacggtaaatggcccgcctggcattatgcccagtacatgaccttatgggactttcctacttggcagtacatctacgtattagtcatcgctattaccatggtgatgcggttttggcagtacatcaatgggcgtggatagcggtttgactcacggggatttccaagtctccaccccattgacgtcaatgggagtttgttttggcaccaaaatcaacgggactttccaaaatgtcgtaacaactccgccccattgacgcaaatgggcggtaggcgtgtacggtgggaggtctatataagcagagctctctggctaactagagaacccactgcttactggcttatcgaaattaatacgactcactatagggagacccaagctgtctagatgccaccatgggctggagcctgatcctcctgttcctcgtcgctgtggctacaggtaaggggctcacagtagcaggcttgaggtctggacatatatatgggtgacaatgacatccactttgcctttctctccacaggtggcgcgcatgccgaaatcaatggctcggccgatcataggatgttttcatttcacaatggaggtgtacagatttcttgtaaataccctgagactgtccagcagttaaaaatgcgattgttcagagagagagaagtcctctgcgaactcaccaagaccaagggaagcggaaatgcggtgtccatcaagaatccaatgctctgtctatatcatctgtcaaacaacagcgtctcttttttcctaaacaacccagacagctcccagggaagctattacttctgcagcctgtccatttttgacccacctccttttcaagaaaggaaccttagtggaggatatttgcatatttatgaatcccagctctggctagcggttgtaagccttgcatatgtacagtcccagaagtatcatctgtcttcatcttccccccaaagcccaaggatgtgctcaccattactctgactcctaaggtcacgtgtgttgtggtagacatcagcaaggatgatcccgaggtccagttcagctggtttgtagatgatgtggaggtgcacacagctcagacgaaaccccgggaggagcagatcaacagcactttccgttcagtcagtgaacttcccatcatgcaccaggactggctcaatggcaaggagttcaaatgcagggtcaacagtgcagctttccctgcccccatcgagaaaaccatctccaaaaccaaaggcagaccgaaggctccacaggtgtacaccattccacctcccaaggagcagatggccaaggataaagtcagtctgacctgcatgataacaaacttcttccctgaagacattactgtggagtggcagtggaatgggcagccagcggagaactacaagaacactcagcccatcatggacacagatggctcttacttcgtctacagcaagctcaatgtgcagaagagcaactgggaggcaggaaatactttcacctgctctgtgttacatgagggcctgcacaaccaccatactgagaagagcctctcccactctcctggtaaaactagtggcaaaccaatcccaaacccactgctgggcctggatagtacttaaaagcttaaacccgctgatcagcctcgactgtgccttctagttgccagccatctgttgtttgcccctcccccgtgccttccttgaccctggaaggtgccactcccactgtcctttcctaataaaatgaggaaattgcatcgcattgtctgagtaggtgtcattctattctggggggtggggtggggcaggacagcaagggggaggattgggaagacaatagcaggcatgctggggatgcggtgggctctatggcttctgaggcggaaagaaccagctggggctctagggggtatccccacgcgccctgtagcggcgcattaagcgcggcgggtgtggtggttacgcgcagcgtgaccgctacacttgccagcgccctagcgcccgctcctttcgctttcttcccttcctttctcgccacgttcgccggctttccccgtcaagctctaaatcgggggctccctttagggttccgatttagtgctttacggcacctcgaccccaaaaaacttgattagggtgatggttcacgtagtgggccatcgccctgatagacggtttttcgccctttgacgttggagtccacgttctttaatagtggactcttgttccaaactggaacaacactcaaccctatctcggtctattcttttgatttataagggattttgccgatttcggcctattggttaaaaaatgagctgatttaacaaaaatttaacgcgaattaattctgtggaatgtgtgtcagttagggtgtggaaagtccccaggctccccagcaggcagaagtatgcaaagcatgcatctcaattagtcagcaaccaggtgtggaaagtccccaggctccccagcaggcagaagtatgcaaagcatgcatctcaattagtcagcaaccatagtcccgcccctaactccgcccatcccgcccctaactccgcccagttccgcccattctccgccccatggctgactaattttttttatttatgcagaggccgaggccgcctctgcctctgagctattccagaagtagtgaggaggcttttttggaggcctaggcttttgcaaaaagctcccgggagcttgtatatccattttcggatctgatcagcacgtgatgaaaaagcctgaactcaccgcgacgtctgtcgagaagtttctgatcgaaaagttcgacagcgtctccgacctgatgcagctctcggagggcgaagaatctcgtgctttcagcttcgatgtaggagggcgtggatatgtcctgcgggtaaatagctgcgccgatggtttctacaaagatcgttatgtttatcggcactttgcatcggccgcgctcccgattccggaagtgcttgacattggggaattcagcgagagcctgacctattgcatctcccgccgtgcacagggtgtcacgttgcaagacctgcctgaaaccgaactgcccgctgttctgcagccggtcgcggaggccatggatgcgatcgctgcggccgatcttagccagacgagcgggttcggcccattcggaccgcaaggaatcggtcaatacactacatggcgtgatttcatatgcgcgattgctgatccccatgtgtatcactggcaaactgtgatggacgacaccgtcagtgcgtccgtcgcgcaggctctcgatgagctgatgctttgggccgaggactgccccgaagtccggcacctcgtgcacgcggatttcggctccaacaatgtcctgacggacaatggccgcataacagcggtcattgactggagcgaggcgatgttcggggattcccaatacgaggtcgccaacatcttcttctggaggccgtggttggcttgtatggagcagcagacgcgctacttcgagcggaggcatccggagcttgcaggatcgccgcggctccgggcgtatatgctccgcattggtcttgaccaactctatcagagcttggttgacggcaatttcgatgatgcagcttgggcgcagggtcgatgcgacgcaatcgtccgatccggagccgggactgtcgggcgtacacaaatcgcccgcagaagcgcggccgtctggaccgatggctgtgtagaagtactcgccgatagtggaaaccgacgccccagcactcgtccgagggcaaaggaatagcacgtgctacgagatttcgattccaccgccgccttctatgaaaggttgggcttcggaatcgttttccgggacgccggctggatgatcctccagcgcggggatctcatgctggagttcttcgcccaccccaacttgtttattgcagcttataatggttacaaataaagcaatagcatcacaaatttcacaaataaagcatttttttcactgcattctagttgtggtttgtccaaactcatcaatgtatcttatcatgtctgtataccgtcgacctctagctagagcttggcgtaatcatggtcatagctgtttcctgtgtgaaattgttatccgctcacaattccacacaacatacgagccggaagcataaagtgtaaagcctggggtgcctaatgagtgagctaactcacattaattgcgttgcgctcactgcccgctttccagtcgggaaacctgtcgtgccagctgcattaatgaatcggccaacgcgcggggagaggcggtttgcgtattgggcgctcttccgcttcctcgctcactgactcgctgcgctcggtcgttcggctgcggcgagcggtatcagctcactcaaaggcggtaatacggttatccacagaatcaggggataacgcaggaaagaacatgtgagcaaaaggccagcaaaaggccaggaaccgtaaaaaggccgcgttgctggcgtttttccataggctccgcccccctgacgagcatcacaaaaatcgacgctcaagtcagaggtggcgaaacccgacaggactataaagataccaggcgtttccccctggaagctccctcgtgcgctctcctgttccgaccctgccgcttaccggatacctgtccgcctttctcccttcgggaagcgtggcgctttctcatagctcacgctgtaggtatctcagttcggtgtaggtcgttcgctccaagctgggctgtgtgcacgaaccccccgttcagcccgaccgctgcgccttatccggtaactatcgtcttgagtccaacccggtaagacacgacttatcgccactggcagcagccactggtaacaggattagcagagcgaggtatgtaggcggtgctacagagttcttgaagtggtggcctaactacggctacactagaagaacagtatttggtatctgcgctctgctgaagccagttaccttcggaaaaagagttggtagctcttgatccggcaaacaaaccaccgctggtagcggtttttttgtttgcaagcagcagattacgcgcagaaaaaaaggatctcaagaagatcctttgatcttttctacggggtctgacgctcagtggaacgaaaactcacgttaagggattttggtcatgagattatcaaaaaggatcttcacctagatccttttaaattaaaaatgaagttttaaatcaatctaaagtatatatgagtaaacttggtctgacagttaccaatgcttaatcagtgaggcacctatctcagcgatctgtctatttcgttcatccatagttgcctgactccccgtcgtgtagataactacgatacgggagggcttaccatctggccccagtgctgcaatgataccgcgagacccacgctcaccggctccagatttatcagcaataaaccagccagccggaagggccgagcgcagaagtggtcctgcaactttatccgcctccatccagtctattaattgttgccgggaagctagagtaagtagttcgccagttaatagtttgcgcaacgttgttgccattgctacaggcatcgtggtgtcacgctcgtcgtttggtatggcttcattcagctccggttcccaacgatcaaggcgagttacatgatcccccatgttgtgcaaaaaagcggttagctccttcggtcctccgatcgttgtcagaagtaagttggccgcagtgttatcactcatggttatggcagcactgcataattctcttactgtcatgccatccgtaagatgcttttctgtgactggtgagtactcaaccaagtcattctgagaatagtgtatgcggcgaccgagttgctcttgcccggcgtcaatacgggataataccgcgccacatagcagaactttaaaagtgctcatcattggaaaacgttcttcggggcgaaaactctcaaggatcttaccgctgttgagatccagttcgatgtaacccactcgtgcacccaactgatcttcagcatcttttactttcaccagcgtttctgggtgagcaaaaacaggaaggcaaaatgccgcaaaaaagggaataagggcgacacggaaatgttgaatactcatactcttcctttttcaatattattgaagcatttatcagggttattgtctcatgagcggatacatatttgaatgtatttagaaaaataaacaaataggggttccgcgcacatttccccgaaaagtgccacctgacgtc

SEQ ID NO: 11 - DNA, 9 bp, artificial
  Kozak sequence
ccaccatgg

SEQ ID NO: 12 - DNA, 41 bp, artificial
  secretory leader sequence
gctggagcctgatcctcctgttcctcgtcgctgtggctaca

SEQ ID NO: 13 - DNA, 84 bp, artificial
  mini intron seq
ggtaaggggctcacagtagcaggcttgaggtctggacatatatatgggtgacaatgacatcctttgcctttctctccacaggtg

SEQ ID NO: 14 - DNA, 42 bp, artificial
  tag sequence
ggcaaaccaatcccaaacccactgctgggcctggatagtact

SEQ ID NO: 15 - DNA, 32 bp, artificial
  primer
ttggcgcgcatgccgaaatcaatggttctgcc

SEQ ID NO: 16 - DNA, 31 bp, artificial
  primer
ctagctagcaagttgtgattcataaatatgc

SEQ ID NO: 17 - DNA, 29 bp, artificial
  primer
ttggcgcgcatgccgaaatcaatggctcg

SEQ ID NO: 18 - DNA, 29 bp, artificial
  primer
ctagctagctagccagagcttcagctggc

SEQ ID NO: 19 - DNA, 18 bp, artificial
  primer
ctgcttactggcttatcg

SEQ ID NO: 20 - DNA, 18 bp, artificial
  primer
cagatggctggcaactag

SEQ ID NO: 21 - DNA, 25 bp, artificial
  siRNA B7h
cagcagccuucgagcugauacucag

SEQ ID NO: 22 - DNA, 25 bp, artificial
  siRNA B7h
cugaguaucagcucgaaggcugcug

SEQ ID NO: 23 - DNA, 25 bp, artificial
  siRNA B7h
ggcccaacguguacuggaucaauaa

SEQ ID NO: 24 - DNA, 25 bp, artificial
  siRNA B7h
uuauugauccaguacacguugggcc